European Patent Application EP 4 674 947 A1, published January 7, 2026. Title: 糖脂質高生産性酵母変異株. Applicant: 花王株式会社. The sequence listing filed with the application follows.

SEQUENCE LISTING (52 sequences)

SEQ ID NO: 1 - DNA, 2184 bp, Starmerella bombicola
  source 1..2184: mol_type = genomic DNA
atgagtttctctcggccgccgacgcagccgcaggggggtgctccctctcaagaaagctcgcctattgccacgcagcccagcgggggtctgccgctacttatgagcagcctctcgcagctcacgcagcagcagcagcagcagcacccacccgcagggcccaacggacagcatcccaatggcccatctagccagaatagccagcttcagcatagccaacctctggcaggacagcctcaacccgggcagacggcacagactgcagcaggcccagcaggccagcagccacatcctggccatgcgtttgggcactccggaccgcttccgcaggcaccaagccagttgggccagttaggagctgctgcagtcgctgctgtgtcgttcccccctcccgcaccgacggcaccattagagatgccacagctgcctcaggtgccctcacggttggtagacttgctggacgggatcaagaatgaatttgcgacaatgagcgcagagacgtcgcgtctgcttttgtctaagcacgatgcagaggcaaagcgtgtgcaggcgcacatggctgagctttcgcaagttcgtaagatcattcaagatcttgacgtcgcgcaccgccagatgcgcgagcgctacgaaagcgagatcgggcgcttgagacagcggctggatgctcttgagccgcagccgccactgctttcgcaaatttcgcaatccgatgagcctgcagaccgccagggacttcctttgccctctcagagtcagccaagctcacaggctcccagccagtcgagctcgcaagtccccagccagcaaatttcgaccctcaacttgccccagcagccaattgtggggccgattcagccgctgccatcgttcgcgcagactcaaccagctcagcctccaagtgctccagcggttagccagagcagtgatcagggcggtcctcccaccccccctgcaggtctcgcaacgccgccattgcccaatgttcctagctcaattgcaaatccagtcagctccgcggccaacctagcgaatttgccggcacaaactgcaccgacaaacgctggagggactggcttcgcgtctgaggattatggctatggtcagaatcttggtagcagcaacagctatgttgatgcgggcaaagttgtgaaaaccgcacgcttagccagcctagatctcgaaaagctgccggcgaaattcaagaaggacgctgatggttatcgagtggtgtacaaccccgaacgtgagccacgactggatgtcgaactgcttcggacactgcaacattcgtcggtagtatgctgtgtgcgcttcagtttagatggtcgcttccttgcgaccggttgcaatcgctcagctcagatttacgatgtcgccacaggcgacctgctgtaccgtttccaagacccgaatgttgacgagagcgtcgatctctacattcgctcggtgtgcttctcgccagacggcaagctgctggcaactggcgccgaggaccacaaggttcgcgtgtgggatatagagaagcgcgagattcgtcacattttcagcggccatgagcaagacatatactcactagcttatgcttccagcggcaaattcattgtttctggcagcggtgaccgcaaggtcaagctttgggacatggagaccgcacagtgccacaaagaattcgttatagacgacggtgtcacagcggtcgctctcagtccagatgaccggtttgtagcagtcggctcgctcgacaagtcagttcgcgtgtgggatgtggaaacgcgcgagctcgtcgagaatctcaacggtgccgacggccatgaggactcagtctactcagtctcatatcgcccagaaggtcgtgagctggtcagtggatctcttgacaaaacccttaaagtgtgggggctgtcttacacgggccagaagcacgagggtcgcgtccggcgcactatcaagggccacaatgactatgtcctttctgttgccgtcactccagactcacattggattttgtcagggtccaaagaccgcactgttcagatgtgggacgccaagactggtgaggtgcagctcatgctgatggcccacgtcaactcggtcattagcgttgcgcagtgcccagtcggtaatctctttgcctcgggcggcggcgatttttcggcaaaaatatggaaatacaccgaggtgtaa

SEQ ID NO: 2 - protein, 727 aa, Starmerella bombicola
MSFSRPPTQPQGGAPSQESSPIATQPSGGLPLLMSSLSQLTQQQQQQHPPAGPNGQHPNGPSSQNSQLQHSQPLAGQPQPGQTAQTAAGPAGQQPHPGHAFGHSGPLPQAPSQLGQLGAAAVAAVSFPPPAPTAPLEMPQLPQVPSRLVDLLDGIKNEFATMSAETSRLLLSKHDAEAKRVQAHMAELSQVRKIIQDLDVAHRQMRERYESEIGRLRQRLDALEPQPPLLSQISQSDEPADRQGLPLPSQSQPSSQAPSQSSSQVPSQQISTLNLPQQPIVGPIQPLPSFAQTQPAQPPSAPAVSQSSDQGGPPTPPAGLATPPLPNVPSSIANPVSSAANLANLPAQTAPTNAGGTGFASEDYGYGQNLGSSNSYVDAGKVVKTARLASLDLEKLPAKFKKDADGYRVVYNPEREPRLDVELLRTLQHSSVVCCVRFSLDGRFLATGCNRSAQIYDVATGDLLYRFQDPNVDESVDLYIRSVCFSPDGKLLATGAEDHKVRVWDIEKREIRHIFSGHEQDIYSLAYASSGKFIVSGSGDRKVKLWDMETAQCHKEFVIDDGVTAVALSPDDRFVAVGSLDKSVRVWDVETRELVENLNGADGHEDSVYSVSYRPEGRELVSGSLDKTLKVWGLSYTGQKHEGRVRRTIKGHNDYVLSVAVTPDSHWILSGSKDRTVQMWDAKTGEVQLMLMAHVNSVISVAQCPVGNLFASGGGDFSAKIWKYTEV

SEQ ID NO: 3 - DNA, 1558 bp, synthetic construct
  source 1..1558: mol_type = other DNA
gttgttgctggagtctcatctgcaaggttgagtaccaatccctgccccaatacgagcaatcgaagccttggggaaagatgcggcgggctagcttcagcaataaatagcaggcgacacacaaaaattaggcggcaagcgcacgctcagcatgccatctaccagggcaaaaagcaaggcaacctctttttcgcatcccgatttagagcctacccgtcattgcagggtgtgcgtctacgatataacacgatcgacatcgcgctgggtatgcttctgggtaaggggtcgcaacgtgtgagttgtcagcactggccgatacccaaagtatataatgcgccgttgaacggttatagtcggtcaagctcttaaagaaagacttaacaacaaaaacaactctacacaaatgaaaaagcctgaactcaccgcgacgtctgtcgagaagtttctgatcgaaaagttcgacagcgtctccgacctgatgcagctctcggagggcgaagaatctcgtgctttcagcttcgatgtaggagggcgtggatatgtcctgcgggtaaatagctgcgccgatggtttctacaaagatcgttatgtttatcggcactttgcatcggccgcgctcccgattccggaagtgcttgacattggggaattcagcgagagcctgacctattgcatctcccgccgtgcacagggtgtcacgttgcaagacctgcctgaaaccgaactgcccgctgttctgcagccggtcgcggaggccatggatgcgatcgctgcggccgatcttagccagacgagcgggttcggcccattcggaccgcaaggaatcggtcaatacactacatggcgtgatttcatatgcgcgattgctgatccccatgtgtatcactggcaaactgtgatggacgacaccgtcagtgcgtccgtcgcgcaggctctcgatgagctgatgctttgggccgaggactgccccgaagtccggcacctcgtgcacgcggatttcggctccaacaatgtcctgacggacaatggccgcataacagcggtcattgactggagcgaggcgatgttcggggattcccaatacgaggtcgccaacatcttcttctggaggccgtggttggcttgtatggagcagcagacgcgctacttcgagcggaggcatccggagcttgcaggatcgccgcggctccgggcgtatatgctccgcattggtcttgaccaactctatcagagcttggttgacggcaatttcgatgatgcagcttgggcgcagggtcgatgcgacgcaatcgtccgatccggagccgggactgtcgggcgtacacaaatcgcccgcagaagcgcggccgtctggaccgatggctgtgtagaagtactcgccgatagtggaaaccgacgccccagcactcgtccgagggcaaaggaataggggagatgggggaggctaactgaaacacggaaggagacaataccggaaggaacccgcgctatgacggcaataaaaagacagaataaaacgcacgggtgttgggtcgtttgttcaaatcactagtatacccgg

SEQ ID NO: 4 - DNA, 26 bp, synthetic construct
  source 1..26: mol_type = other DNA
gttgttgctggagtctcatctgcaag

SEQ ID NO: 5 - DNA, 27 bp, synthetic construct
  source 1..27: mol_type = other DNA
ccgggtatactagtgatttgaacaaac

SEQ ID NO: 6 - DNA, 45 bp, synthetic construct
  source 1..45: mol_type = other DNA
gccaagcttgcatgcttgggcaccttctgcgcacccagcacggag

SEQ ID NO: 7 - DNA, 48 bp, synthetic construct
  source 1..48: mol_type = other DNA
gactccagcaacaaccattaatatcgagcttggctcctaatactatac

SEQ ID NO: 8 - DNA, 43 bp, synthetic construct
  source 1..43: mol_type = other DNA
cactagtatacccggacttcgtatatggccaggctgccttgag

SEQ ID NO: 9 - DNA, 39 bp, synthetic construct
  source 1..39: mol_type = other DNA
agagtcgacctgcagcaatgacgatagcgaagatcccac

SEQ ID NO: 10 - DNA, 25 bp, synthetic construct
  source 1..25: mol_type = other DNA
gcatgcaagcttggcactggccgtc

SEQ ID NO: 11 - DNA, 27 bp, synthetic construct
  source 1..27: mol_type = other DNA
ctgcaggtcgactctagaggatccccg

SEQ ID NO: 12 - DNA, 20 bp, synthetic construct
  source 1..20: mol_type = other DNA
ctcttcgctattacgccagc

SEQ ID NO: 13 - DNA, 20 bp, synthetic construct
  source 1..20: mol_type = other DNA
cactttatgcttccggctcg

SEQ ID NO: 14 - DNA, 23 bp, synthetic construct
  source 1..23: mol_type = other DNA
ttgggcaccttctgcgcacccag

SEQ ID NO: 15 - DNA, 21 bp, synthetic construct
  source 1..21: mol_type = other DNA
caatgacgatagcgaagatcc

SEQ ID NO: 16 - DNA, 21 bp, synthetic construct
  source 1..21: mol_type = other DNA
cttgactgagcgctcaagaag

SEQ ID NO: 17 - DNA, 21 bp, synthetic construct
  source 1..21: mol_type = other DNA
ggtgcagccaaccactaattc

SEQ ID NO: 18 - DNA, 3996 bp, synthetic construct
  source 1..3996: mol_type = other DNA
tataggtcaatagagtatacttatttgtcctattgattagatagcagtataatagctttatagagtaggtcatttaagttgagcataataggtcatttttttgattttttttaattttatatcacattaataagcctaaattatcgcgtatgtatgtgcaaagccggctgaggtacataatacggccgaatggtctagttggttatggcgctagtctaacactcgttagttcactggaggtccccagttcgatcctgggttcggtcaattcttttttgtccaaaatctcgacagctctcagttcaaggcgaccttaacctcaaatcgccaacccgttttttttgtatcttattcacagggttgttggcctggcttatgaaccagtggaaaagaatacttggggtactcagcttgctctcggttgcaattgctatgagcgtgtttgttccttccaacgagtggcaatttgtgcccgagaacgtggccataccggggggtctagaagtcaagttagaccttgagaaaggaggacggtgggcgagaatattgcaagataacggtagagaagaccagaaattagcagagcgcctcacagaatcgactccctctacatatgacctggcgactgtcactcttgactccgcacaactagaagcaatggaagagaaggctcacgactacgacgacggagcagatatcgctcgacttcacggactcaccttgttcaacctatttaaagatacgagcgacccagcccacgatcaagccggtagaatcctcagtatctgcatgagaaataacaatgacgccacaagagccgtagcaacgatgtgccccaacctgtcacaagctttaaagtttgaccggagatcgctatcgattgtgagcgccctagtatccaaccccgaggggcgaaaatacttgcagagccatggcgcattggacaaggtccgccgcgaccttgccacagccgatcagatcgacagcaccacaagcacagcgatttcaaagcttgtacaagatctggcgatcgctggagaagactctgaagacttctgtaaatgggtcgacgccttgcaacaagcttattacaccactcaaaatccaacactgaaacagcttgctatcgacatagtccaacataatggcgaatttgaatcgctaactgtcgaatgcaggccccagcctgggttgttgcctccgcatgaggagcataagagggccgaggaatctgctcgtcgctttgaaaatcgattggcttcacgaaaccattttgatgagttatgagaattcttggagatcgaatttgccgatcgtttcgtgaatgcgagcttagaagccctcatcgccctaaagcttttcattatttccagaatagggtaagtcgcgctcagcttgagcgtggggaaatggcctattaagggcgttaagctgcagaaaagatccgccctacttccaaacctcgccctggatactgatccccacaattcttaagctgcgaggtgttcagacaagcgcccttcatagcgctaggacagcaaagtagccgaaactggtatatttgggagatcagttgaaacaaacaaagctcttttgtcatggccaagatcggctacgcccgcgtcagctccaaggaacagaacctggaccgccaactccaggccctccagggcgtcagcaaggtgttctccgacaagctgtccggccagtccgtcgagcgcccccagctccaggccatgctgaactacatccgcgagggcgacatcgtcgtcgtcaccgagctggaccgcctgggccgcaacaacaaggaactgaccgagctgatgaacgccatccagcagaagggcgccaccctcgaggtcctgaacctgccctccatgaacggcatcgaggacgagaacctgcgccgcctgatcaacaacctggtcatcgagctgtacaagtaccaggccgagtccgagcgcaagcgcatcaaggaacgccaggcccagggcatcgagatcgccaagtccaagggcaagttcaagggccgccagcacaagttcaaggaaaacgacccccgcctgaagcacgccttcgacctgttcctcaacggctgctccgacaaggaagtcgaggaacagaccggcatcaaccgccgcaccttccgccgctaccgcacccgctacaacgtcaccgtcgaccagcgcaagaacaagggcaagcgcgactcctgagggagatgggggaggctaactgaaacacggaaggagacaataccggaaggaacccgcgctatgacggcaataaaaagacagaataaaacgcacgggtgttgggtcgtttgttcaaatcactagtatacccgggttgttgctggagtctcatctgcaaggttgagtaccaatccctgccccaatacgagcaatcgaagccttggggaaagatgcggcgggctagcttcagcaataaatagcaggcgacacacaaaaattaggcggcaagcgcacgctcagcatgccatctaccagggcaaaaagcaaggcaacctctttttcgcatcccgatttagagcctacccgtcattgcagggtgtgcgtctacgatataacacgatcgacatcgcgctgggtatgcttctgggtaaggggtcgcaacgtgtgagttgtcagcactggccgatacccaaagtatataatgcgccgttgaacggttatagtcggtcaagctcttaaagaaagacttaacaacaaaaacaactctacacaaatgaaaaagcctgaactcaccgcgacgtctgtcgagaagtttctgatcgaaaagttcgacagcgtctccgacctgatgcagctctcggagggcgaagaatctcgtgctttcagcttcgatgtaggagggcgtggatatgtcctgcgggtaaatagctgcgccgatggtttctacaaagatcgttatgtttatcggcactttgcatcggccgcgctcccgattccggaagtgcttgacattggggaattcagcgagagcctgacctattgcatctcccgccgtgcacagggtgtcacgttgcaagacctgcctgaaaccgaactgcccgctgttctgcagccggtcgcggaggccatggatgcgatcgctgcggccgatcttagccagacgagcgggttcggcccattcggaccgcaaggaatcggtcaatacactacatggcgtgatttcatatgcgcgattgctgatccccatgtgtatcactggcaaactgtgatggacgacaccgtcagtgcgtccgtcgcgcaggctctcgatgagctgatgctttgggccgaggactgccccgaagtccggcacctcgtgcacgcggatttcggctccaacaatgtcctgacggacaatggccgcataacagcggtcattgactggagcgaggcgatgttcggggattcccaatacgaggtcgccaacatcttcttctggaggccgtggttggcttgtatggagcagcagacgcgctacttcgagcggaggcatccggagcttgcaggatcgccgcggctccgggcgtatatgctccgcattggtcttgaccaactctatcagagcttggttgacggcaatttcgatgatgcagcttgggcgcagggtcgatgcgacgcaatcgtccgatccggagccgggactgtcgggcgtacacaaatcgcccgcagaagcgcggccgtctggaccgatggctgtgtagaagtactcgccgatagtggaaaccgacgccccagcactcgtccgagggcaaaggaataggggagatgggggaggctaactgaaacacggaaggagacaataccggaaggaacccgcgctatgacggcaataaaaagacagaataaaacgcacgggtgttgggtcgtttgttcaaatcactagtatacccggtataggtcaatagagtatacttatttgtcctattgattagatagcagtataatagctttatagagtaggtcatttaagttgagcataata

SEQ ID NO: 19 - DNA, 42 bp, synthetic construct
  source 1..42: mol_type = other DNA
tccggaattgacacatataggtcaatagagtatacttatttg

SEQ ID NO: 20 - DNA, 42 bp, synthetic construct
  source 1..42: mol_type = other DNA
taaatctagatgatatattatgctcaacttaaatgacctact

SEQ ID NO: 21 - DNA, 26 bp, synthetic construct
  source 1..26: mol_type = other DNA
gcatgcaagcttggcactggccgtcg

SEQ ID NO: 22 - DNA, 26 bp, synthetic construct
  source 1..26: mol_type = other DNA
ctgcaggtcgactctagaggatcccc

SEQ ID NO: 23 - DNA, 42 bp, synthetic construct
  source 1..42: mol_type = other DNA
gccaagcttgcatgcgaaggggctctccgaagtacatcactg

SEQ ID NO: 24 - DNA, 42 bp, synthetic construct
  source 1..42: mol_type = other DNA
tgtgtcaattccggaaaaacgacagaaaagtgctgaggccgc

SEQ ID NO: 25 - DNA, 42 bp, synthetic construct
  source 1..42: mol_type = other DNA
tatcatctagatttatatcacaagtcactatttacttgttta

SEQ ID NO: 26 - DNA, 42 bp, synthetic construct
  source 1..42: mol_type = other DNA
agagtcgacctgcagctcaatgaactgagacagcagcttgtc

SEQ ID NO: 27 - DNA, 20 bp, synthetic construct
  source 1..20: mol_type = other DNA
ctcttcgctattacgccagc

SEQ ID NO: 28 - DNA, 20 bp, synthetic construct
  source 1..20: mol_type = other DNA
cactttatgcttccggctcg

SEQ ID NO: 29 - DNA, 21 bp, synthetic construct
  source 1..21: mol_type = other DNA
gaaggggctctccgaagtaca

SEQ ID NO: 30 - DNA, 21 bp, synthetic construct
  source 1..21: mol_type = other DNA
ctcaatgaactgagacagcag

SEQ ID NO: 31 - DNA, 21 bp, synthetic construct
  source 1..21: mol_type = other DNA
ctaaggccagtacaagagatc

SEQ ID NO: 32 - DNA, 26 bp, synthetic construct
  source 1..26: mol_type = other DNA
ctaaagctcgaattaatagagacacg

SEQ ID NO: 33 - DNA, 1815 bp, Starmerella bombicola
  source 1..1815: mol_type = genomic DNA
atgacggaagaggaggtccaacaggtatttcttggttttgtgcattctcgcattggttccttgagaatgtttgccacaggaatcaccagccttgctcttttagttgcctacagagtgtccccggagttgcgcaagactctcggggatgctgacacgcaccctcatcttcttagtatcaaggcaaaaatcaatacaaaagaggttatttggcatctgcccaaattcgcaatcccccctcctctaagtccaaatcagcctgcagcgataaccacggatgttgtgattgttggttccggttgctcaagtatggtggcttcttatcttttgacaaagaagggtttcaatgtgatcattgtggaaaaaggctaccacatcaatgcaattaccagtcccgaacacgacttccaacgtgacatcgaggcgtttgagggtgaacacaatatgacatctgcggatgcctcaacaatagttgttgcgggcgccacggtcggaggcggtggtgcagttaactggagctgttccttacgtccaactgagcttgttagacgtgagtttgtccagaaaggagctccactctatggctcgaaagagtttgaccacgctttggctgaggtcgaacgggttatgcaagtaagcactaagttcggtcttgagggtggcagcgataacgaacattcattcacgaacgatttgatcttgaaggccagcgagaagctcaattatcgagccaaggtcgcaggtcaaaatactgggaagcacagagcaaactctggcttcgtcgagtttggcagcagacagggcgaggctgaaggcggggtcgctgagtggttccgcaacagtttcaacaacggtgctcggttgctgcagagaggccacgttgtcaacatcaggcaccataacggttacgcctctggtgtagaggtagttgtagacgggtcaaagaccattttgataaactgcaaacgagttgtgtgcgctgcagggtcacttcagactccagtgctgctgcagaggtcaggtttcaagaactctcatatcggcaagggcctgaaattgcacccggtcactgcagcttatggtgtcttccccgaacagatagtgaacaagcgacttgatcccattatgaccacggtttgcacagaagtcgacaatctcgacggtgaaggccacgggccaaagatcgaggcgctgcaccacaggcctcttctcacatccttccctctgccataccgcgatgccaaggactttcaaaccaaggtggagagctgggagcatctttgcacgcttctggtcatcactcgtgataagggagaaggcaaagtgagcttttatcccccgaatccctcaaagccttatatcgaatacacgccgagcaagtatgatcttggggctctgctgaaagggtccctgtctgctgcgaacatgctttacgtacaaggcgcgcaacgcatattcttgtcaagcacattcatccccgatttcgtatccaataagccggtatctgagcgatcaatttgggacgacgactatcagaaatggtaccaggaggccaagcgcaaggaattcattctatatgacactaaagttgggtctgctcatcaaatgggtacctgtcgcatgagcgtgaacgggcccaagcatggcgccgttgacggaaagggacacctttacgagtgccccaatgttcacgttattgatacttcggtgtttcccgctgcttcgggcgtcaatccgatgataacgtgcatggctactgcttacgtgcttgcaaacaatcttatcgcggatctcactaagcttcaaactaagctatga

SEQ ID NO: 34 - protein, 604 aa, Starmerella bombicola
MTEEEVQQVFLGFVHSRIGSLRMFATGITSLALLVAYRVSPELRKTLGDADTHPHLLSIKAKINTKEVIWHLPKFAIPPPLSPNQPAAITTDVVIVGSGCSSMVASYLLTKKGFNVIIVEKGYHINAITSPEHDFQRDIEAFEGEHNMTSADASTIVVAGATVGGGGAVNWSCSLRPTELVRREFVQKGAPLYGSKEFDHALAEVERVMQVSTKFGLEGGSDNEHSFTNDLILKASEKLNYRAKVAGQNTGKHRANSGFVEFGSRQGEAEGGVAEWFRNSFNNGARLLQRGHVVNIRHHNGYASGVEVVVDGSKTILINCKRVVCAAGSLQTPVLLQRSGFKNSHIGKGLKLHPVTAAYGVFPEQIVNKRLDPIMTTVCTEVDNLDGEGHGPKIEALHHRPLLTSFPLPYRDAKDFQTKVESWEHLCTLLVITRDKGEGKVSFYPPNPSKPYIEYTPSKYDLGALLKGSLSAANMLYVQGAQRIFLSSTFIPDFVSNKPVSERSIWDDDYQKWYQEAKRKEFILYDTKVGSAHQMGTCRMSVNGPKHGAVDGKGHLYECPNVHVIDTSVFPAASGVNPMITCMATAYVLANNLIADLTKLQTKL

SEQ ID NO: 35 - DNA, 3618 bp, Starmerella bombicola
  source 1..3618: mol_type = genomic DNA
atgacagatttcggaacccgcatagagcacactttcacatccggattcgaagggctcaggcgtcagtcaggatcccaattcgaacacattcagcttcacgactcgccttctcccaatcccgcagtcgctgattttagcgctcattccacttgcatggaggattcggcagctgccggtggtgcaaatcccaaggttccaagcaccgaagaactccaaaaggccgcaggtgcacctggtgcagctggtagcgaaccaatccctgccaaatctctggtgattaagacgaaaaagcctaggccatacgcttgtcctacgtgcacacgtagttttgctcgtttggagcatctcaaacggcatgagcgttcccacaccaaggagaaaccgtttcagtgtccggtgtgtgagcgcagctttgctagacgagaccttcttctgcgtcacaagcaaaaactccatgcgtctttctctccaacagaagaaaagcatcaagtcaaggactcacagttcccgggccaagtacctctggaccagggtcctgtccagtcgatcaggcagaccaacactggatcccagcctctcagtcaacatggcctatcacccctaaatgcgagggcaatggctcctgccaacgccatatatgctacctcggcacggttgctggcaaataatcaaacctcgtcgccctctccttccgttggcatgaacatgcaaaaccaaatggcccagctcatgcagaactacgaaggtatggacctgctcactcctcttcgctccacctcaccttcggaagctcaaatgcaaaatatgaatgctatgggtggtttgaacaactcaaacggctacatacctgctacagattcgttcaagcaagtcttccctcagcagacttcgttccctctgatgaactcccgcggtgaaaacaatttcggtgagtggaggcagctcaacccactcgcacacgagctcgaaatgcttcatggtgttgctccctcattcagagcagtctcgaatcgcccctctagagccagctccttcagtgctgcttcagctaccacataccttcgtgagaaggacctaaacttgtacccaacttcgcagcagtttggccaggaggcctcagaggtcggatttgccactcctcaggcgtacgctgtcgatgatgagggctacgatttcgagccattggacctgaacttcgtgtccccagctcagttgagccagccgccgccgcgtaagcgtcgggtgagccttcatacatcttcggcaagtcctatgatgaatgcgttccaagaaggaactccggcgataaacctaaatattcagcctcaaggacaaagccaagggcacctcgattctcctcaaccaggacctgcaatgctggcattgcgggcccaagcacgtacacagagacagctgtaccagaaccaccactttggctcgggaagcgttgagtctccgtcgtcattgagtttcttcgaatccggcgacaccattggcagtctgtcaggagttagccaaagcccatcaccacagcagcaccttgcgaaccagccgcagcagcctccaagtcagcagcctccaagccagcagcctccaagccagcagcaacaaactccgcaaacacagagacagccagcgtccagcaggcaacagtcgttggacagcttgttctctggcttagatagttcgtttggagagttttgtgggtctccaggcatgacgccagggttcacccctgagatggcgtccggaatgacgcctgcttttactcccagcatgcacgccccgtatcagaccagcatgtcgcctcttcctgaggaagccggtgatatcaaagactttatggcacagcagaacgacgacttcgtaaactcattatttgacgccgaaggtaaatcgcccgagctgcgtaaaagcggatactgttctgatagttataccgatagcagtggtttgaatgggagccatagtggcagcgccaatggcagcataaacggaagccacaccgggaatcatagcgaaagtcacaatggaagtcaccacggaaaccccaatggaggttttcatggcggtgtaagcttcgggattaacgatctgggcaacaacactaatagctcaggcagcaatgaggtcagcggaatgcagaggttcatggactcttacttcaacagcttcgatacacatttgtcatttgttcacaaagcctcacaggtctcacatgcgctctctgaattctcatcgaccatcggctctccagccatctctcctccatcttcgtcctcgtctgttggcaccaccgccgacacaagtttgaatgccaagcttgctctctcacaagcactggctgcagttggagcgcaaactttaggagagcgtggtgaagctcaggcatattattgggcagcacgcgaccataacaactcaggaagtaccactttggaagggctgcaggcagacattttagttgcggtacttggtttgttcttcgacgaaccttctgagcatgcagcttctttagataaactcacgtcatcgattacagagacggagttgattatcgctccactaacgaagtcccagaactactcaacttacgatagtggccatggccttggaggcgcccaatctctcaaagtttctgaggagtggccggctaacgctgagaggctttgggaccaatttattgccaaccaatcacgcgtcaggacgctccacgcattgcatgcaatttgctgttgggtgcgcagaccatctcagcagctactaaacgttctagaatcctgtggatgtgctccatgcgatgatgacctatggagagcacccaccagcgacatttggttgcgggtagttgcatcgaaagaactggatgcgcatcaggtcgccgaaacaggaggcaatcctcctcagcagttcagaatggtcttaaataagctgcgaaatggagaggtgccccaggaagttgtatcacagtttacgttacagtcgttactgttagctttagagctttcgtgtgaccctgcagaatactctttgcagtcttctagggcagcattgagggcctgggaaacgctttgggctcgaagcccagatgcctctctcgatcccagtccagagagtgggccgatcatgagtgattgtgtcggaattgtgtcgttggttgcattttcatctctgaaaatgcgtggtgttcttgatgctctgtggcaacatgactttgctaaggtcagtcaagaggtgtccaaggctgtcaagggacagcagtatagcgcctcctcagtcgctaattatgctgtggatactctcgtatggtgtgagggtcatgtttcatcccattcaatcttcttctctacactcctcgctgtttcggagtgtgggctggtgcttgccgagtccctacggctcatcatctcgaaaaacacgccaactagcaacgcagaggagcagcttatccaacgaagcaggaaacttgtgagtacagtgctcaaagtatcgccctctgccgacctcgagatgcttcccaatcacgttctgagagctgctgtgtgcttgattagactgagcgactggcctcttgttggtgctctttctcgcatgctgcttggtcacctgtcgacttga

SEQ ID NO: 36 - protein, 1205 aa, Starmerella bombicola
MTDFGTRIEHTFTSGFEGLRRQSGSQFEHIQLHDSPSPNPAVADFSAHSTCMEDSAAAGGANPKVPSTEELQKAAGAPGAAGSEPIPAKSLVIKTKKPRPYACPTCTRSFARLEHLKRHERSHTKEKPFQCPVCERSFARRDLLLRHKQKLHASFSPTEEKHQVKDSQFPGQVPLDQGPVQSIRQTNTGSQPLSQHGLSPLNARAMAPANAIYATSARLLANNQTSSPSPSVGMNMQNQMAQLMQNYEGMDLLTPLRSTSPSEAQMQNMNAMGGLNNSNGYIPATDSFKQVFPQQTSFPLMNSRGENNFGEWRQLNPLAHELEMLHGVAPSFRAVSNRPSRASSFSAASATTYLREKDLNLYPTSQQFGQEASEVGFATPQAYAVDDEGYDFEPLDLNFVSPAQLSQPPPRKRRVSLHTSSASPMMNAFQEGTPAINLNIQPQGQSQGHLDSPQPGPAMLALRAQARTQRQLYQNHHFGSGSVESPSSLSFFESGDTIGSLSGVSQSPSPQQHLANQPQQPPSQQPPSQQPPSQQQQTPQTQRQPASSRQQSLDSLFSGLDSSFGEFCGSPGMTPGFTPEMASGMTPAFTPSMHAPYQTSMSPLPEEAGDIKDFMAQQNDDFVNSLFDAEGKSPELRKSGYCSDSYTDSSGLNGSHSGSANGSINGSHTGNHSESHNGSHHGNPNGGFHGGVSFGINDLGNNTNSSGSNEVSGMQRFMDSYFNSFDTHLSFVHKASQVSHALSEFSSTIGSPAISPPSSSSSVGTTADTSLNAKLALSQALAAVGAQTLGERGEAQAYYWAARDHNNSGSTTLEGLQADILVAVLGLFFDEPSEHAASLDKLTSSITETELIIAPLTKSQNYSTYDSGHGLGGAQSLKVSEEWPANAERLWDQFIANQSRVRTLHALHAICCWVRRPSQQLLNVLESCGCAPCDDDLWRAPTSDIWLRVVASKELDAHQVAETGGNPPQQFRMVLNKLRNGEVPQEVVSQFTLQSLLLALELSCDPAEYSLQSSRAALRAWETLWARSPDASLDPSPESGPIMSDCVGIVSLVAFSSLKMRGVLDALWQHDFAKVSQEVSKAVKGQQYSASSVANYAVDTLVWCEGHVSSHSIFFSTLLAVSECGLVLAESLRLIISKNTPTSNAEEQLIQRSRKLVSTVLKVSPSADLEMLPNHVLRAAVCLIRLSDWPLVGALSRMLLGHLST

SEQ ID NO: 37 - DNA, 1617 bp, Starmerella bombicola
  source 1..1617: mol_type = genomic DNA
atgttaatcaaagacattattctaactccaatgagtttatccgctgttgctggcttgttgccactgctcttcgtagctttcttagttctacacgagcctatctggctcctatggtaccgctatgcagcacgtaggcacaagtgtagtatgcctcgcttcattgagaaatcgttcccactgggaatacaaagaaccatggacatgatcaagacggccaagtcatacaccttactggaagttcaatacgacagagtcttcaataagttcaaagcacggacgtatcttcgacaagctccccttcaataccaaatcttcacaatcgagccagaaaacattaagacaatcctggcaaccaaattcaatgattttggtcttggagcacgtttccacacagtgggaaaagtgtttggccaagggatatttacactcagcggaaatggatggaaacagtctcgatcgatgttgagacctcagttcactaaagatcaggtttgcagaattgatcagatttccagtcatgctgcggagttaataaaggagatgaaccgtgcaatgaaagtggaccaatttattgatgttcaacattatttccacaaacttacgctggatacagcgactgaattcctatttggggagtcctgcgagagcttgaaccctgagaatcagtcatgtattgtagcccgtgatggttcggagattactgccgaacaattcgtggagtcctacaactttctactgaattacgctttcaaacggaccctatcaagcaaagtctactggttgttcaactctaaggaattccgagatcacaagaaacgtgctcagtcctatattgactactacgttgataaggctctttacgccacatctttcgctgctgagaactctattgcagagaaggatgctgctgcagagtctagtggcatctatgtgttctcgcttgagatggctaaagttacccgagacccagtgacgatacgtgatcaaattttcaacattctcattgctggtagagatacaacagctgctacgttgagcttcgctattcatttccttgccagaaatcctgacgtattcaacaaactacgtgaggaggtcctcgatcattttggaaccaaggaggagcaaaggcctttatcattcgaacttctgaagcaagcaccttatttgaagcaagttataaatgaagtcttgcgtcttgcgccggtattgccattgaacttccgtactgctgtgagagatacaactctacccataggtggtggtcccgagcagaaggatccgatcttcgttcctaagggcaccgcagtttactattcaatttacatggtccacagggacatcaagtattggggtcctgacgcccacgaattcaatcccaatcgatgggagaacttgaagctagataatgtgtgggcattcttgcccttcaatggcggtccccgaatttgtctcggccaacaattcgccctgacagagctttcgctaactctggtgagactcttacaggagtattccaagattgagatgggtcccgacttcccagagtcccctcgtttctcaacaacgcttacagctcaacacgctcctcccggtgtggttgtgcggttttcttaa

SEQ ID NO: 38 - protein, 538 aa, Starmerella bombicola
MLIKDIILTPMSLSAVAGLLPLLFVAFLVLHEPIWLLWYRYAARRHKCSMPRFIEKSFPLGIQRTMDMIKTAKSYTLLEVQYDRVFNKFKARTYLRQAPLQYQIFTIEPENIKTILATKFNDFGLGARFHTVGKVFGQGIFTLSGNGWKQSRSMLRPQFTKDQVCRIDQISSHAAELIKEMNRAMKVDQFIDVQHYFHKLTLDTATEFLFGESCESLNPENQSCIVARDGSEITAEQFVESYNFLLNYAFKRTLSSKVYWLFNSKEFRDHKKRAQSYIDYYVDKALYATSFAAENSIAEKDAAAESSGIYVFSLEMAKVTRDPVTIRDQIFNILIAGRDTTAATLSFAIHFLARNPDVFNKLREEVLDHFGTKEEQRPLSFELLKQAPYLKQVINEVLRLAPVLPLNFRTAVRDTTLPIGGGPEQKDPIFVPKGTAVYYSIYMVHRDIKYWGPDAHEFNPNRWENLKLDNVWAFLPFNGGPRICLGQQFALTELSLTLVRLLQEYSKIEMGPDFPESPRFSTTLTAQHAPPGVVVRFS

SEQ ID NO: 39 - DNA, 1572 bp, Starmerella bombicola
  source 1..1572: mol_type = genomic DNA
atgattctttatgctgtgctgggcgcattcgccgccttcttgctttacatggatgtactttaccctttcgtgatttaccctctgagagcgcgatggcacaaatgtggttacatccctagagatttgagctggccattggggattccactcaccctggtagttctctcgaagttgaggaaagatatgctgctgcaattcatggcagcgcaagaccttagtcgcccttacaagacatccttacgtcaatttctgggtaaatgggtaatcgccactagagatcctgagaacatcaaggctgttctatccaccaagttcaatgacttctcgctgaaagaaagagggaataggatgaggcatgtaatcggtgatggaatttttacccaagatggcgcaccatggaagcactcgcgagatatgctcaggcctcagttcaccaaggatcaaatcagccgagtggaattgttgagccaccacatcgacgttttgattcgtgaaatcaggaagtcgggaggtaacgtcgagttgcaacgtttattccacctcatgactatggacaccgccactcactttctattcggcgagtccgttggctcgttggaggtcagtggcgaaagcaagggcattgagatcaccgacccaaagactggagagattgtgaacaccgttgattttgttgagtcttatacttttgcaaacaagtttgctctcaagaagattatcctcaacgacttggagtttttagccgacttgacggagccctcgtataagtggcatctgcgccgtgtccacacagtcatggatcactacgttcagctggctttgaaggctactgagaagtatgatcctgatgatgatagcgagaagggagaatactactttagccatgagctggcgaaactcacgagagaccccttgtcgttgagagatcagcttttcaatattctcattgctggccgcgacactaccgcagcaactttgtcctatgccttccactatctaacgaagaatcccgctatctacgccaaggtccgcgaagatgtgctcacggtcttccctaatggagacgcatcattggcgacttacgaggacttgcgaaaggctaagtatctccaaatggtgatcaaggaggtattgcgtcttgcgcctgcggttcccttgaacacgcgtgccgcggttcgtgacacatatctgccacggggcggaggcccagccggaaacctgcccgtttttgttcccaagggcactgctgtcaactaccctacatatattttgcaccgcgatccagatatctatggtgccgacgcgtacgagttcaaccccgagagatggaggcctgagaataagcttccgaatagcccaatgtactcttggggatacattcccttcaatggtggccctcgcatctgcattggacagcagttcgccttgactgagatcgctttgacgatgatcaagctggttctggaatttgagaggctggagcctgccgacgactttgagcccaatcttcaagacaagtcctctttaactgtcatggtcggagggtcgggcgtccgagtgaaactgagttaa

SEQ ID NO: 40 - protein, 523 aa, Starmerella bombicola
MILYAVLGAFAAFLLYMDVLYPFVIYPLRARWHKCGYIPRDLSWPLGIPLTLVVLSKLRKDMLLQFMAAQDLSRPYKTSLRQFLGKWVIATRDPENIKAVLSTKFNDFSLKERGNRMRHVIGDGIFTQDGAPWKHSRDMLRPQFTKDQISRVELLSHHIDVLIREIRKSGGNVELQRLFHLMTMDTATHFLFGESVGSLEVSGESKGIEITDPKTGEIVNTVDFVESYTFANKFALKKIILNDLEFLADLTEPSYKWHLRRVHTVMDHYVQLALKATEKYDPDDDSEKGEYYFSHELAKLTRDPLSLRDQLFNILIAGRDTTAATLSYAFHYLTKNPAIYAKVREDVLTVFPNGDASLATYEDLRKAKYLQMVIKEVLRLAPAVPLNTRAAVRDTYLPRGGGPAGNLPVFVPKGTAVNYPTYILHRDPDIYGADAYEFNPERWRPENKLPNSPMYSWGYIPFNGGPRICIGQQFALTEIALTMIKLVLEFERLEPADDFEPNLQDKSSLTVMVGGSGVRVKLS

SEQ ID NO: 41 - DNA, 1671 bp, Starmerella bombicola
  source 1..1671: mol_type = genomic DNA
atgaggcccctgttgcgggaacaagacacatcacacccagagctattgttggcaagcaatactatttttaaccccctttccaagagtgtccaaactgttcaatacggcctcatgaacattaatttctctgacgtgctcgtgctaggaggcatcagcgtgagctttttgctcgcctaccaggcgatttacttttatttcatttactcgccacgagccaaaaagctcggttgcgctcttccaccggtcttcttctctttcccactcggaataccggaggtcatacgtcttgtgaacgcctggttcaacgatgatctccttgagtatttcaccttcaaattcgaggagttccagcgcaaaaccggattccaatcagtcgctgggcaactatggattgggactattgagcccgagaacatcaagactatgctcgctacttcatttaaagactactccctaggcttccgttacgaggccatgtacggccttctcggaaatggcattttcactctcagtggtgagggctggaagcacagccgcgctttgttgcgtccgcaatttagtcgtgagcaagtctctcaccttgaatcaatgcgcacacacatcaatatgttgatcaacaaccacttcaagggtggcaaagtcgtcgatgctcaggttttgttccacaatctaaccattgatactgctaccgaattcctattcggagagagcaccaacactcttgaccctgctcttgctcagcatggattccctggacctaagggtcttgtaaccggtgagcagtttgctgaggcttttacctctgctctcgaattgctttctgtgcgagttatggccggcgccgcatggttcctcgtttggacccccaaattctggcgctcatgcaaagtctgccacaacttcattgattacttcgttttcaaggctctggccactcctatggagaaggaccaggaagctgatcgctacgtctttattcgagaactcacaaaggagacctctgacccacgggtcatccgcgaccaggccctcaacatcctcttggctggtcgtgataccactgcggcacttctcagcttcaccacctactaccttggtgcctaccctgaggtctacgatgagcttcgcgaggctgttattgcggacttcggcaaggaagatgctgagccccctacgtttgagcagcttaagcagtgcaaggtgctacagaacgtcattcgggaagttttgcgattgcacccgaatgtgcccctcaacttccgcgaggccattaccgatactaagttccccacaggaggcggcccgaatggagaccagcccgttttcgttcccaagggacagaaagtgttttacgccacctacgtcatgcagcgaaatgagggtctctggggtcctgactccacaacattccgccctgaccgctggaacgagtcaagagaggccatcgcatccggatgggactacattcctttcaacggcggccctcgtatttgcctgggtcagcagttcgctctcacagaggcgagctacacgctcgtgcgtatctgccaagagttctccaggattgaggttctccaccctgatgttattacctccaggaacgtgatgaaacagcgcatgcgtttgaccaactcttccagcggcggcgtcatagcgaagttcattcgctag

SEQ ID NO: 42 - protein, 556 aa, Starmerella bombicola
MRPLLREQDTSHPELLLASNTIFNPLSKSVQTVQYGLMNINFSDVLVLGGISVSFLLAYQAIYFYFIYSPRAKKLGCALPPVFFSFPLGIPEVIRLVNAWFNDDLLEYFTFKFEEFQRKTGFQSVAGQLWIGTIEPENIKTMLATSFKDYSLGFRYEAMYGLLGNGIFTLSGEGWKHSRALLRPQFSREQVSHLESMRTHINMLINNHFKGGKVVDAQVLFHNLTIDTATEFLFGESTNTLDPALAQHGFPGPKGLVTGEQFAEAFTSALELLSVRVMAGAAWFLVWTPKFWRSCKVCHNFIDYFVFKALATPMEKDQEADRYVFIRELTKETSDPRVIRDQALNILLAGRDTTAALLSFTTYYLGAYPEVYDELREAVIADFGKEDAEPPTFEQLKQCKVLQNVIREVLRLHPNVPLNFREAITDTKFPTGGGPNGDQPVFVPKGQKVFYATYVMQRNEGLWGPDSTTFRPDRWNESREAIASGWDYIPFNGGPRICLGQQFALTEASYTLVRICQEFSRIEVLHPDVITSRNVMKQRMRLTNSSSGGVIAKFIR

SEQ ID NO: 43 - DNA, 1299 bp, Starmerella bombicola
  source 1..1299: mol_type = genomic DNA
atggccatcgagaaaccagtgatagttgcttgtgcctgcccactagcggggcacgtgggcccagtgctcagcctggtccgcggtctactcaatagaggatatgaggtgactttcgtaacagggaacgcattcaaggagaaagttattgaggcaggatgcactttcgtccctctccaaggacgagctgactaccatgaatacaatctccctgaaatcgctccaggattgctcacgattcctccaggccttgagcagaccggttactcaatgaatgagatttttgtgaaggcgattcctgagcagtacgatgcacttcaaactgctctaaaacaggttgaggctgaaaataaatcagctgtggtgattggcgagaccatgtttctaggggtgcatccgatatcactgggtgccccaggtctcaagccccaaggcgtaatcacgttaggaactattccgtgcatgctgaaagcagagaaggcgcctggagttcctagtcttgagccaatgattgatactttagtgcggcaacaagtatttcaaccaggaactgactctgagaaggagatcatgaagacgctcggggccacgaaggagcccgaatttctcctggagaatatatacagcagccctgacagatttttgcaactgtgccctccatctcttgaatttcacttgacttcgcctcctcctggcttctcgttcgctggtagtgcaccgcatgtaaagtctgctggattagcaactccacctcacctgccgtcttggtggcctgatgtgctgagtgcgaagcgtctgattgttgttacacaaggaacagcagccatcaactatgaagatctgctcattccagcattgcaggcctttgctgacgaagaagacactctcgtagttggtatattgggcgtcaaaggggcgtcacttcctgatagcgttaaagttcctgcaaacgctcgaattgttgattattttccttacgatgagctactaccgcatgcctctgttttcatatacaacggtggatacggaggtctgcagcacagtttgagccatggcgttcccgtcatcatcggaggaggaatgttggtagacaagccagctgttgcttcacgagctgtatgggctggtgttggttatgatcttcaaaccttgcaggcaacttctgagctagtctccacggccgttaaggaggtgttggctactccctcgtatcacgagaaagccatggcagtcaagaaagagcttgaaaaatacaagtctcttgatattctagagtcggcaattagtgaattagcttcttaa

SEQ ID NO: 44 - protein, 432 aa, Starmerella bombicola
MAIEKPVIVACACPLAGHVGPVLSLVRGLLNRGYEVTFVTGNAFKEKVIEAGCTFVPLQGRADYHEYNLPEIAPGLLTIPPGLEQTGYSMNEIFVKAIPEQYDALQTALKQVEAENKSAVVIGETMFLGVHPISLGAPGLKPQGVITLGTIPCMLKAEKAPGVPSLEPMIDTLVRQQVFQPGTDSEKEIMKTLGATKEPEFLLENIYSSPDRFLQLCPPSLEFHLTSPPPGFSFAGSAPHVKSAGLATPPHLPSWWPDVLSAKRLIVVTQGTAAINYEDLLIPALQAFADEEDTLVVGILGVKGASLPDSVKVPANARIVDYFPYDELLPHASVFIYNGGYGGLQHSLSHGVPVIIGGGMLVDKPAVASRAVWAGVGYDLQTLQATSELVSTAVKEVLATPSYHEKAMAVKKELEKYKSLDILESAISELAS

SEQ ID NO: 45 - DNA, 1392 bp, Starmerella bombicola
  source 1..1392: mol_type = genomic DNA
atgagcccttcatcacacaaacccctgattctcgcttgcggcttgcctctttcaggccatataatgcccgttttgagtctggtacacggccttacggacgacggatacgaagctactgttgtgacaggcagagcgtttgaacaaaaagttcgagatgtgggtgcagactttgttcctttagaagggaacgcagattttgatgaccacaccttagacgatctggtcccgggccgtaaagacatggccccaagcttcgatcgtacagttcaagatgtggagcacatgatggtagctactcttcctgagcagtttgccgctattcagagggctttcaaaaagctcagcgcaagcggccgccctgtcgttcttgtcagtgaagtgctgtttttcggtgcacaccctatcagcctcggtgctcctggtttcaaacccgctggctggatttgtttaggggttttgcctcttttgatccgcagtgatcataccttaggacttgacaacgacaggagccccgaagcacatgcaaagaaactcgctatgaaccacgctcttgagcaccaaattttcgttaaagccactgctaagcacaaggaaatctgccgagagttaggttgcactgaagatcccaaatttatctgggagcacagttacattgctgcagacaagttcctgcagctgtgcccgccttctcttgagttcagcagagaccatctgcctagcaacttcaaattcgccggctcaacgcccaagcaccgaactcaattcacccctccttcctggtggggggatgttctgagtgccaagcgagtcatcatggtcactcaaggaacttttgctgtcagttacaagcatcttattgtgcctactcttgaggccttgaaggacgagcctgacactttaacagtagccatattgggccgccgcggtgccaagctaccggatgatgttgtggttcctgagaatgctcgcgtgatcgactacttcaactacgatgctctacttcctcacgttgatgctcttgtctacaatggtggatatggcggacttcagcacagcttaagccactctgttccagttgttattgctggtgactctgaagacaagccaatggtggcatcgagagctgaggccgctggcgtggcaattgatttgaaaactggcttgcctacagtggagcaaatcaaagaagctgttgattcgataattggaaatccgaaattccacgaagcctcgaagaaggttcaaatggagttggaaagccacaactccttgaaaattcttgaggaaagcatcgaggaaatcgccagccatgactttggtcttttgaccaagagtgacgaggaaactgaagatatacctgtcaaagggccggccttagcggtgagttcttag

SEQ ID NO: 46 - protein, 463 aa, Starmerella bombicola
MSPSSHKPLILACGLPLSGHIMPVLSLVHGLTDDGYEATVVTGRAFEQKVRDVGADFVPLEGNADFDDHTLDDLVPGRKDMAPSFDRTVQDVEHMMVATLPEQFAAIQRAFKKLSASGRPVVLVSEVLFFGAHPISLGAPGFKPAGWICLGVLPLLIRSDHTLGLDNDRSPEAHAKKLAMNHALEHQIFVKATAKHKEICRELGCTEDPKFIWEHSYIAADKFLQLCPPSLEFSRDHLPSNFKFAGSTPKHRTQFTPPSWWGDVLSAKRVIMVTQGTFAVSYKHLIVPTLEALKDEPDTLTVAILGRRGAKLPDDVVVPENARVIDYFNYDALLPHVDALVYNGGYGGLQHSLSHSVPVVIAGDSEDKPMVASRAEAAGVAIDLKTGLPTVEQIKEAVDSIIGNPKFHEASKKVQMELESHNSLKILEESIEEIASHDFGLLTKSDEETEDIPVKGPALAVSS

SEQ ID NO: 47 - DNA, 780 bp, Starmerella bombicola
  source 1..780: mol_type = genomic DNA
atggttgtaaactcctcgaaggaccctcaaaacaaaggaatgactcctagaaaagaaattgaccaggaaatggtctcttgggccaaaaaaaacctcaaaaacacccctggcaatgaaaactatgagaagatggtctcaggagttccttacaatccatacgatccagatcttatgtttagagccctggctactagtgagaaagttagggagttcaataccattgcaagtgaaagtcgtacttttgagtcaaatcacgctgcttatatcaagaaggtcgagattctcaaagacacttttggtcaaacaaaggatattgtctggctgaccgctccattctcagttgattttggattcaacatcagcgtaggcgagcacttttacgccaacttcaacgtttgcttcttggactcggctccaataatctttggtgatgaggtgattgtagggcccaatacaacgttcgtgactgcgactcatcctattagccccgagaaacgtgcgaggagaattgtgtatgctcttcctatcaaggtggggaataatgtatggattggtgcgaatgtgactgtcctgccgggtgttacgattggagatggctcaacaattgcggctggtgctgtcgttcgagaagatgttcctcctcgtactgtggtgggaggagtccctgcgcgaatcctcaagcatattccagaggaggatcccgacgaggctgaaggagaggaactggaattccttcttccagttgaaatgaacgtcaataccgctaaccagaaggtctag

SEQ ID NO: 48 - protein, 259 aa, Starmerella bombicola
MVVNSSKDPQNKGMTPRKEIDQEMVSWAKKNLKNTPGNENYEKMVSGVPYNPYDPDLMFRALATSEKVREFNTIASESRTFESNHAAYIKKVEILKDTFGQTKDIVWLTAPFSVDFGFNISVGEHFYANFNVCFLDSAPIIFGDEVIVGPNTTFVTATHPISPEKRARRIVYALPIKVGNNVWIGANVTVLPGVTIGDGSTIAAGAVVREDVPPRTVVGGVPARILKHIPEEDPDEAEGEELEFLLPVEMNVNTANQKV

SEQ ID NO: 49 - DNA, 1233 bp, Starmerella bombicola
  source 1..1233: mol_type = genomic DNA
atgctggctctgtttttttcgcttgcgcctctactttctcaagctctccctttaggctatactgcggcccccgctgaatcattctatttttggccagagaacatatccagcctccaagctggcgagatttttagaaaacgggaactcttaactctcccagacatctttgactttggccctaatctggaaaaggtcgtacaagtggcttacaaaacccgtctcaccgatggcaatgactcgttttccatcgccagtatctttatccctaagaatccaagcccagaactcaaactttactcttatcagacgtttgaggatgccgtgcagcttgattgtgccccaagctatgctttagaagtgggtaacaagtccagcaactatcttcctgtcactagcaatttatctgccatcagtcgagaacttgagaaaggacgtcactgcattatccctgatcacgagggctatatttcaggattctttgcaggacggcaggagggatatgctggtttagacggaattcgcgctgctcgaaactatctcaatggcaccaacgagaccccaattggtatcttcggatacagtggaggtgcacaagcaacggcctggattgttgatttgcatgacgagtatgctcctgacttgaactttgttggaacagtttctggaggcactttggttgacgcttggggcacttttcagtatatcgactatccgaaggtgtatctaaagggcagcattcttatcatgtatacgggtcttttttcaggttatccagctcaatttgaggtgatttggccatatattgagcctgtaattcaagaaaacatgctactgctacgtttggcgccgaatgattgtaaccaaagcccgatacttcaaggttacaacaattcaatcatggccggtatacatgtggaccttcccgaattccctgcttctaagtacatattccagcacgagtccctccttgccaactacagcgtagtgccagtttccacaccgaagtttcctcgctacatgtaccatggtggatctgatgagttggccaaattgagccttgtcgagcagtatgttgatcaacaatggaataccggcgctaatctcaccttcgtggtgtatccgggtcttcttcatgacgagacggcttaccgtggctttgatgccgcgatggattggcttgatgcccagctcgatagtggataccttccacctgtaaactcaactcatacatga

SEQ ID NO: 50 - protein, 410 aa, Starmerella bombicola
MLALFFSLAPLLSQALPLGYTAAPAESFYFWPENISSLQAGEIFRKRELLTLPDIFDFGPNLEKVVQVAYKTRLTDGNDSFSIASIFIPKNPSPELKLYSYQTFEDAVQLDCAPSYALEVGNKSSNYLPVTSNLSAISRELEKGRHCIIPDHEGYISGFFAGRQEGYAGLDGIRAARNYLNGTNETPIGIFGYSGGAQATAWIVDLHDEYAPDLNFVGTVSGGTLVDAWGTFQYIDYPKVYLKGSILIMYTGLFSGYPAQFEVIWPYIEPVIQENMLLLRLAPNDCNQSPILQGYNNSIMAGIHVDLPEFPASKYIFQHESLLANYSVVPVSTPKFPRYMYHGGSDELAKLSLVEQYVDQQWNTGANLTFVVYPGLLHDETAYRGFDAAMDWLDAQLDSGYLPPVNSTHT

SEQ ID NO: 51 - DNA, 3900 bp, Starmerella bombicola
  source 1..3900: mol_type = genomic DNA
atggtggatgatatacaggtagagaagcgtgagaaactcatcgagactaaggacaagcttctcgaggagaagctctctgcgttagatccacatgaggccaatgtattgcgaagtcagcttgaaacaaagagagtcgccacaagctttttcaggttgttcagattttgcactccccttgacgttttcttggagatacttgcgcttttttttgcagcggtgcatggagccgcgcttccaatgttcacgttagtagtgggcgccatcttcaacacattcagagacttcacttcatatgacctcaagggcaatgagttccagcataaggtgaatcacctgtctctctattttgtctatattggcattggtatgctcggcagtgcgtttctcgagagcttcctgcttgtggacagaggcgaagtgttggcaggacgttaccgaaagcattatctgagtgctgttattcgccagaatatcgcgttttacgacaaactaggtggtggcgaggtcagcaccagaatcattaacgataccaactcaattcaggaagcgatcagcgacaagcttggaaacgtcgtacagggaatagcttccttcattgcggccaccgttataagttttgcttcgcaatggaaactggcttgcatcctcctgagtgctgtagggttcatggtaatcacaatgggaactggcgccaccttcatggccaaatatcagctcagatctgacgcgatatattcgcagtctggagctaccgttgcggaggaggctctcagtgctgtcaggactacagtagcatttggcgctcaacctcatctcgccgtcaagtatgaaaaggtacttgatcgtgttgtgaaggaatcgaagcggagcagttactcattgggggtcatgttagcgtgcatatgggctagtactttttgggtgtatgccttagctctgtggcagggttccagagaaatcgttagtgggagtgctgacgttggaaagataatagttgtaatcacagctatgttacttggaagcttccagcttgggaatatcgcgccaaacgtgaggtttcttgtcaagggtctcactgccgcgagcattctcaatgaggccattgatcgtgtcccagtcatcgatggccagtccatagataaaggaattgtcccccaaactaaggccgttggcagaattgagctcaaaaatgtcaagttccgatatcctagtcgcccagacgttttggtcctctccgattttagccttgaagttcctgctggatctactgtggcactggtaggtgcctcgggatcagggaagtctacaattgtaggtattcttgagaggttctatttacctctcgaaggaagcgttactctggatggccaggagattagcgacctgaacacaagatggctccgtcaacaaattggttatgttcagcaggaaccagtactcttttcagagtcaatatatgagaatatcagctatggtttgattggcactgacattgagttcgctgacgagcatgttaaggaagctaaaatcattcaagcttgtaaagatgccaatgcctgggatttcattcagactctctcagaaggcatccaaaccaatgttggagatcgaggatttcttctcagcggtggtcagaaacaacgcattgcaatagcaagagcaatcgtctcagaccctaaaattctgctgctcgatgaagcgacttctgctctggataccaaatctgaaggtatcgttcaagatgcgctcgacaaagcggccgaaggtcgtaccactatagtcgttgcacacagactctctacgatcaaggatgccaacaagatagttgtcatgtctaaaggtaacgtcatagagcagggtactcacaatgagctcatacagcgagaagggccttataaagctttggttgatgctcaaagagtaactaaagcaaagagcactaacgttgaggtcctcgatattgaagctctagacatttcgcctctggactcactgaacgaaaagttcaatcccaaggatgtgagcacattgagtgttcacagtgcaggtactcagaccactcaacctcctgaatatcaagaaaatgacatccctggtgtgcgcaaccccccacatagcacgttgatgaccaataccaaactggtttgggggctgaataggaaagaatggggttacattctcattggtagtttagcctccattattttgggctattgctatcctgcaatggcaataataactggccaaaccactggaagcatggttctacctcccagtgaatacggaaaaatgcggcatgtggtgaatatcatgggatggtggtattttttcgtaggctgcatttcattcatgacggcttttatcactatagctgctttatcacttgcatctgataagttggtcaaaaatatcagattagctttgttccgccaattgatgcgaatggatattgcattcttcgaccacaaaaacaacacgccgggtgcgctaacctcaattttggcgaaggaagctaaaatgatcgagggtttgagtggggccaccctcggtcaaattcaacagagtctggtgaccttgattggcggcatagttactggtatacctttcaattggagaattggactcgtggctacgtctgttgttcctgtcatgttggtgtgtggcttcgtcagagtctgggttcttacccaattatcggatcgtgcgagagaagtttacgaacgaagtggctccatggcatctgagtatacaagtgctgtccgcacagtccagtccttaactcgtgagttagacgtggtcgtaaaatacacaaagacagtagactctcagattttcagctccagaattgccattgcccgctcagcattgtactacgcactctcggaaggaatgacaccctgggtggtagccctcgttttttggtggggaagcactgtaatgagacgaggtgaagcttcggtcgcaggatatatgactgtcttcatggctattattacaggttctcaagccgctggccaaattttcagctatgctccaaacatgaactcagccaaagatgcagcgcgtaacatttacagaatcttgactgccactccttctatagatgtatggagtgaggaaggttacgttgctcccgaggagtcggtgagaggagatattgagttccgtcatgtgaatttccgatatcctactcgacctcaagtaccagttttacaagatctcaacttaacagtcaaaaagggccaatacatcgctctagttggagccagtggatgcggtaagtctactactattggactggtggaaagattttatgatccattagcaggtcaagtacttttcgatgggaaagatttacgcgaatataacctgaatgcattgagatcacacattgctttagtccagcaagaaccaatgctttattcaggcacgctacgtgagaatattctaatgggatggtctggccctgagtctgaagtaacgcaggagatgattgaggatgccgctcgcaaagcgaacattcacgaattcatcatgtcgttgcctgatggctacgaaacgctcagcggatctaggggatcgttgctatctggggggcaaaagcagcgaattgcaattgcaagggccctgatcagaaatccaaaggtactcctcctcgatgaggccacctcagctctggattccgaatctgagaaagtagttcaagcagcactcgacgcagcagcgaagggccgtactacaatcgccgttgcgcatagattatcaacaattcagaaagcagatgtcatatatgtgttctcaggagggcgcatcgtggagcagggcgaccatcagagcctccttgaactcaatggatggtacgctgaattggtgaacttgcaaggtctcggagagatttga

SEQ ID NO: 52 - protein, 1299 aa, Starmerella bombicola
MVDDIQVEKREKLIETKDKLLEEKLSALDPHEANVLRSQLETKRVATSFFRLFRFCTPLDVFLEILALFFAAVHGAALPMFTLVVGAIFNTFRDFTSYDLKGNEFQHKVNHLSLYFVYIGIGMLGSAFLESFLLVDRGEVLAGRYRKHYLSAVIRQNIAFYDKLGGGEVSTRIINDTNSIQEAISDKLGNVVQGIASFIAATVISFASQWKLACILLSAVGFMVITMGTGATFMAKYQLRSDAIYSQSGATVAEEALSAVRTTVAFGAQPHLAVKYEKVLDRVVKESKRSSYSLGVMLACIWASTFWVYALALWQGSREIVSGSADVGKIIVVITAMLLGSFQLGNIAPNVRFLVKGLTAASILNEAIDRVPVIDGQSIDKGIVPQTKAVGRIELKNVKFRYPSRPDVLVLSDFSLEVPAGSTVALVGASGSGKSTIVGILERFYLPLEGSVTLDGQEISDLNTRWLRQQIGYVQQEPVLFSESIYENISYGLIGTDIEFADEHVKEAKIIQACKDANAWDFIQTLSEGIQTNVGDRGFLLSGGQKQRIAIARAIVSDPKILLLDEATSALDTKSEGIVQDALDKAAEGRTTIVVAHRLSTIKDANKIVVMSKGNVIEQGTHNELIQREGPYKALVDAQRVTKAKSTNVEVLDIEALDISPLDSLNEKFNPKDVSTLSVHSAGTQTTQPPEYQENDIPGVRNPPHSTLMTNTKLVWGLNRKEWGYILIGSLASIILGYCYPAMAIITGQTTGSMVLPPSEYGKMRHVVNIMGWWYFFVGCISFMTAFITIAALSLASDKLVKNIRLALFRQLMRMDIAFFDHKNNTPGALTSILAKEAKMIEGLSGATLGQIQQSLVTLIGGIVTGIPFNWRIGLVATSVVPVMLVCGFVRVWVLTQLSDRAREVYERSGSMASEYTSAVRTVQSLTRELDVVVKYTKTVDSQIFSSRIAIARSALYYALSEGMTPWVVALVFWWGSTVMRRGEASVAGYMTVFMAIITGSQAAGQIFSYAPNMNSAKDAARNIYRILTATPSIDVWSEEGYVAPEESVRGDIEFRHVNFRYPTRPQVPVLQDLNLTVKKGQYIALVGASGCGKSTTIGLVERFYDPLAGQVLFDGKDLREYNLNALRSHIALVQQEPMLYSGTLRENILMGWSGPESEVTQEMIEDAARKANIHEFIMSLPDGYETLSGSRGSLLSGGQKQRIAIARALIRNPKVLLLDEATSALDSESEKVVQAALDAAAKGRTTIAVAHRLSTIQKADVIYVFSGGRIVEQGDHQSLLELNGWYAELVNLQGLGEI